European Patent Specification EP 2 968 347 B1, published August 2, 2023. Title: Modulators of the eIF2alpha  Pathway. Applicant: Walter, Peter Sidrauski, Carmela Acosta-Alvear, Diego Arkin, Michelle R. Wilson, Christopher G. Ang, Kean-Hooi Hearn, Brian R. Vedantham, Punitha Renslo, Adam R. Maze, Mervyn Vacas, Susana. The sequence listing filed with the application follows.

SEQUENCE LISTING (14 sequences)

SEQ ID NO: 1 - DNA, 19 bp, Artificial Sequence
  Synthetic polynucleotide
gtagcctgatggggtgctt

SEQ ID NO: 2 - DNA, 18 bp, Artificial Sequence
  Synthetic polynucleotide
tgaggcagccggagatac

SEQ ID NO: 3 - DNA, 20 bp, Artificial Sequence
  Synthetic polynucleotide
agccaaaatcagagctggaa

SEQ ID NO: 4 - DNA, 20 bp, Artificial Sequence
  Synthetic polynucleotide
tggatcagtctggaaaagca

SEQ ID NO: 5 - DNA, 20 bp, Artificial Sequence
  Synthetic polynucleotide
tggaagatggtgatgggatt

SEQ ID NO: 6 - DNA, 19 bp, Artificial Sequence
  Synthetic polynucleotide
agccacatcgctcagacac

SEQ ID NO: 7 - DNA, 20 bp, Artificial Sequence
  Synthetic polynucleotide
gaagccaaggggaatgaagt

SEQ ID NO: 8 - DNA, 20 bp, Artificial Sequence
  Synthetic polynucleotide
gagatgttctggaggggtga

SEQ ID NO: 9 - DNA, 26 bp, Artificial Sequence
  Synthetic polynucleotide
  misc_feature (1)..(1): 5'-terminal modified with FAM
  misc_feature (26)..(26): 3'-terminal modified with BHQ1
cagcactcagactacgtgcacctctg

SEQ ID NO: 10 - DNA, 24 bp, Artificial Sequence
  Synthetic polynucleotide
  misc_feature (1)..(1): 5'-terminal modified with HEX
  misc_feature (24)..(24): 3'-terminal modified with BHQ1
tctgctgagtccgcagcaggtgca

SEQ ID NO: 11 - DNA, 20 bp, Artificial Sequence
  Synthetic polynucleotide
actgggtccaagttgtccag

SEQ ID NO: 12 - DNA, 20 bp, Artificial Sequence
  Synthetic polynucleotide
ggagttaagacagcgcttgg

SEQ ID NO: 13 - DNA, 20 bp, Artificial Sequence
  Synthetic polynucleotide
tggaagatggtgatgggatt

SEQ ID NO: 14 - DNA, 19 bp, Artificial Sequence
  Synthetic polynucleotide
agccacatcgctcagacac